European Patent Application EP 4 711 466 A1, published March 18, 2026. Title: 工程化的mRNA及其用途. Applicant: 北京先声祥瑞生物制品股份有限公司. Application CN. The sequence listing filed with the application follows.

SEQUENCE LISTING (22 sequences)

SEQ ID NO: 1 - RNA, 60 nt, Artificial Sequence
  source 1..60: mol_type = other RNA
ggataaaagacttcagacaccacaaacgaattagccacgataaccccccccgacgccacc

SEQ ID NO: 2 - RNA, 60 nt, Artificial Sequence
  source 1..60: mol_type = other RNA
gggacccgacacgcatcacaacacctatcaaagcaaaccgacaacgcaccacacgccacc

SEQ ID NO: 3 - RNA, 60 nt, Artificial Sequence
  source 1..60: mol_type = other RNA
gggaaaactttacacgacacgagagcatcagacgacaggaccataaacacaaccgccacc

SEQ ID NO: 4 - RNA, 60 nt, Artificial Sequence
  source 1..60: mol_type = other RNA
gggaacacagacaagaactcacgaacacctagcaccatacaccaacgacaatacgccacc

SEQ ID NO: 5 - RNA, 70 nt, Artificial Sequence
  source 1..70: mol_type = other RNA
gggaaaaatacacacgatcacacctaagcagaaaaaccaatccaaccaaccgaccacaacgcacgccacc

SEQ ID NO: 6 - RNA, 60 nt, Artificial Sequence
  source 1..60: mol_type = other RNA
ggatacacgcataccacgagagcttacgacaacaacaacattaattgacccgacgccacc

SEQ ID NO: 7 - RNA, 60 nt, Artificial Sequence
  source 1..60: mol_type = other RNA
ggaagaacgacaattgacgcaccatagacgaccgaaataatcccgaccacatttgccacc

SEQ ID NO: 8 - RNA, 60 nt, Artificial Sequence
  source 1..60: mol_type = other RNA
gggacaacgagcagcacacgaagatacacaacagaaaggagaaatcacactagcgccacc

SEQ ID NO: 9 - RNA, 60 nt, Artificial Sequence
  source 1..60: mol_type = other RNA
ggaacaaggaatacacaggagacgacggaacgaaggacacagacgataacaagagccacc

SEQ ID NO: 10 - RNA, 49 nt, Artificial Sequence
  source 1..49: mol_type = other RNA
ggaggaacagcaaattcaggaaaaagtggcgacctttcgactcgccacc

SEQ ID NO: 11 - RNA, 295 nt, Artificial Sequence
  source 1..295: mol_type = other RNA
ctcgagctggtactgcatgcacgcaatgctagctgcccctttcccgtcctgggtaccccgagtctcccccgacctcgggtcccaggtatgctcccacctccacctgccccactcaccacctctgctagttccagacacctcccaagcacgcagcaatgcagctcaaaacgcttagcctagccacacccccacgggaaacagcagtgattaacctttagcaataaacgaaagtttaactaagctatactaaccccagggttggtcaatttcgtgccagccacaccctggagctagc

SEQ ID NO: 12 - RNA, 110 nt, Artificial Sequence
  source 1..110: mol_type = other RNA
aaaaaaaaaaaaaaaaaaaaaaaaaaaaaagcatatgactaaaaaaaaaaaaaaaaaaaaaaaaaaaaaaaaaaaaaaaaaaaaaaaaaaaaaaaaaaaaaaaaaaaaaa

SEQ ID NO: 13 - DNA, 88 bp, Artificial Sequence
  source 1..88: mol_type = other DNA
gggtcggcatggcatctccacctcctcgcggtccgacctgggcatccgaaggaggacgcacgtccactcggatggctaagggagggcg

SEQ ID NO: 14 - DNA, 720 bp, Artificial Sequence
  source 1..720: mol_type = other DNA
atggtgagcaagggcgaggagctgttcaccggggtggtgcccatcctggtcgagctggacggcgacgtaaacggccacaagttcagcgtgtccggcgagggcgagggcgatgccacctacggcaagctgaccctgaagttcatctgcaccaccggcaagctgcccgtgccctggcccaccctcgtgaccaccctgacctacggcgtgcagtgcttcagccgctaccccgaccacatgaagcagcacgacttcttcaagtccgccatgcccgaaggctacgtccaggagcgcaccatcttcttcaaggacgacggcaactacaagacccgcgccgaggtgaagttcgagggcgacaccctggtgaaccgcatcgagctgaagggcatcgacttcaaggaggacggcaacatcctggggcacaagctggagtacaactacaacagccacaacgtctatatcatggccgacaagcagaagaacggcatcaaggtgaacttcaagatccgccacaacatcgaggacggcagcgtgcagctcgccgaccactaccagcagaacacccccatcggcgacggccccgtgctgctgcccgacaaccactacctgagcacccagtccgccctgagcaaagaccccaacgagaagcgcgatcacatggtcctgctggagttcgtgaccgccgccgggatcactctcggcatggacgagctgtacaagtga

SEQ ID NO: 15 - RNA, 57 nt, Artificial Sequence
  source 1..57: mol_type = other RNA
gggaaataagagagaaaagaagagtaagaagaaatataagaccccggcgccgccacc

SEQ ID NO: 16 - RNA, 45 nt, Artificial Sequence
  source 1..45: mol_type = other RNA
gggcgcgcctagcagtgtcccagccgggttcgtgtcgccgccacc

SEQ ID NO: 17 - RNA, 41 nt, Artificial Sequence
  source 1..41: mol_type = other RNA
gggactcttctggtccccacagactcagagagaacgccacc

SEQ ID NO: 18 - RNA, 70 nt, Artificial Sequence
  source 1..70: mol_type = other RNA
ggcaaaaatcaaaatcaatcatcatcacaacatcaacaatcaatcatcaacacatcatcaagacaccacc

SEQ ID NO: 19 - RNA, 54 nt, Artificial Sequence
  source 1..54: mol_type = other RNA
gagaataaactagtattcttctggtccccacagactcagagagaacccgccacc

SEQ ID NO: 20 - DNA, 771 bp, Artificial Sequence
  source 1..771: mol_type = other DNA
atggtcccctgcacactgctgctgctgctggccgccgcactggctccaactcagactcgggcacgaaccgtccctccaatggtcaacgtgacccggtctgaggccagcgagggcaacatcaccgtgacatgccgggccagctccttctaccctagaaatatcatcctgacatggaggcaggacggcgtgtccctgtctcacgatacccagcagtggggcgacgtgctgccagatggcaacggcacctaccagacatgggtggcaaccaggatctgcaggggcgaggagcagaggttcacatgttatatggagcacagcggcaatcactccacccacccagtgccctctggcaaggtgctggtgctgcagagccactggcagacatttcacggcggcggcggctctggaggaggaggaagcggaggaggaggctcccgcaccgtgccccctatggtgaacgtgacatgctccgaggtgtctgagggcaatatcaccgtgacatgtcgcgcctctagcttctatccccggaacatcaccctgacatggagacaggacggcgtgagcctgtcccacaacactcagcagtggggagacgtgctgcctgatggcaatggaacttaccagacatgggtggccacacggatcagacagggcgaggagcagagatttacctgttatatggagcactccggcaatcacggcacccatcccgtcccctctggcaaagccctggtcctgcagtctcagcgaaccgatttcccctgataatag

SEQ ID NO: 21 - DNA, 771 bp, Artificial Sequence
  source 1..771: mol_type = other DNA
atggtcccttgcacactgctgctgctgctggctgctgccctggctccaactcagactcgcgcccgaaccgtccctccaatggtccaggtgacacggtctgaggccagcgagggccagatcaccgtgacatgccgggccagctccttctaccctagaaacatcatcctgacatggaggcaggacggcgtgtccctgtctcacgatacccagcagtggggagacgtgctgccagatggacagggcacctaccagacatgggtggcaaccaggatctgcaggggcgaggagcagaggttcacatgttatatggagcacagcggacagcactccacccacccagtgccctctggcaaggtgctggtgctgcagagccactggcagacctttcacggaggaggaggatctggaggaggaggaagcggcggaggaggctcccgcaccgtgccccctatggtgcaggtgacatgctccgaggtgtctgaaggacagatcaccgtgacatgtcgcgcctctagcttctatccccggaacatcaatctgacatggagacaggacggcgtgagcctgtcccacaacactcagcagtggggcgatgtgctgcctgacggccagggaacttaccagacatgggtggccacacggatcagacagggcgaggagcagagatttacctgttatatggagcactccggccagcacggcacccaccccgtcccaagcggcaaagccctggtcctgcagtcacagcgaacagatttcccttgataatag

SEQ ID NO: 22 - DNA, 1305 bp, Artificial Sequence
  source 1..1305: mol_type = other DNA
atggtcccttgtaccctgctgctgctgctggctgctgccctggccccaactcagactcgcgctcgcactgtcccacctatggtcaacgtgacccggtccgaggcctctgagggcaacatcaccgtgacatgccgggccagctccttctacccaagaaatatcatcctgacctggaggcaggacggcgtgtctctgagccacgatacacagcagtggggagacgtgctgccagatggaaacggcacctaccagacatgggtggcaaccaggatctgcaggggcgaggagcagcggttcacatgttatatggagcactctggcaatcacagcacccacccagtgccatccggaaaggtgctggtgctgcagtctcactggcagacctttcacggaggaggaggatccggaggaggaggatctggcggcggcggcagcagaaccgtgccccctatggtgaacgtgacatgcagcgaggtgtccgagggcaatatcaccgtgacatgtcgcgcctctagcttttatcctcggaacatcaccctgacatggagacaggacggcgtgtccctgtctcacaacacccagcagtggggcgacgtgctgccagatggcaatggaacttaccagacatgggtggccacacggatcagacagggcgaggagcagaggttcacctgctatatggagcacagcggcaatcacggcacacaccctgtgccaagcggaaaggccctggtgctgcagtcccagaggaccgactttccaggcggcggcggcagcggcggcggcggctccggcggcggcggcagcgatatcatcaagctgctgaacgagcaagtgaataaggagatgcagtcctctaacctgtacatgtctatgagctcctggtgttatacacactccctggacggagcaggcctgttcctgtttgatcacgccgccgaggagtacgagcacgccaagaagctgatcatcttcctgaatgagaacaatgtgcccgtgcagctgatcagcatctccgcccctgagcacaagttcgagggcctgacccagatctttcagaaggcctacgagcacgagcagcacatctctgagagcatcaacaatatcgtggaccacgccatcaagtccaaggatcacgccacattcaactttctgcagtggtacgtggccgagcagcacgaggaggaggtgctgtttaaggacatcctggataagatcgagctgatcggcaatgagaaccacggcctgtacctggcagaccagtatgtcaagggaatcgcaaagtcacgcaaaagctgataatag